European Patent Specification EP 2 913 392 B1, published June 7, 2023. Title: 組換え細胞、並びに、イソプレンの生産方法. Applicant: Sekisui Chemical Co., Ltd. The sequence listing filed with the application follows.

SEQUENCE LISTING (20 sequences)

SEQ ID NO: 1 - DNA, 1788 bp, Populus nigra
  CDS (1)..(1788)
atggcaactgaattattgtgcttgcaccgtccaatctcactgacacacaaattgttcagaaatcccttgcctaaagtcatccaggccactcccttaactttgaaactcagatgttctgtaagcacagaaaacgtcagcttcacagaaacagaaacagaaaccagaaggtctgccaattatgaaccaaatagctgggattatgattatttgctgtcttcggacactgacgaatcgattgaagtatacaaagacaaggccaaaaagctggaggctgaggtgagaagagagattaacaatgaaaaggcagagtttttgactctgcctgaactgatagataatgtccaaaggttaggattaggttaccggttcgagagtgacataaggagagcccttgatagatttgtttcttcaggaggatttgatgctgttacaaaaactagccttcatgctactgctcttagcttcaggcttctcagacagcatggctttgaggtctctcaagaagcgttcagcggattcaaggatcaaaatggcaatttcttgaaaaaccttaaggaggacatcaaggcaatactaagcctatatgaagcttcatttcttgccttagaaggagaaaatatcttggatgaggccaaggtgtttgcaatatcacatctaaaagagctcagcgaagaaaagattggaaaagacctggccgaacaggtgaatcatgcattggagcttccattgcatcgaaggacgcaaagactagaagctgtttggagcattgaagcataccgtaaaaaggaagatgcagatcaagtactgctagaacttgctatattggactacaacatgattcaatcagtataccaaagagatcttcgcgagacatcaaggtggtggaggcgtgtgggtcttgcaacaaagttgcattttgctagagacaggttaattgaaagcttttactgggcagttggagttgcgtttgaacctcaatacagtgattgccgtaattccgtagcaaaaatgttttcgtttgtaacaatcattgatgatatctatgatgtttatggtactctggatgagttggagctatttacagatgctgttgagagatgggatgttaatgccatcgatgatcttccggattatatgaagctctgcttcctagctctctataacactatcaatgagatagcttatgataatctgaaggacaagggggaaaacattcttccatacctaacaaaagcgtgggcagatttatgcaatgcattcctacaagaagcaaaatggttgtacaataagtccacaccaacatttgatgaatatttcggaaatgcatggaaatcatcctcagggcctcttcaactagtttttgcctactttgccgttgttcaaaacatcaagaaagaggaaattgataacttacaaaagtatcatgatatcatcagtaggccttcccacatctttcgtctttgcaacgacttggcttcagcatcggctgagatagcgagaggtgaaaccgcgaattctgtatcatgctacatgcgtacaaaaggcatttctgaggaacttgctactgaatccgtaatgaatttgatcgacgaaacctggaaaaagatgaacaaagaaaagcttggtggctctctgtttgcaaaaccttttgtcgaaacagctattaaccttgcacgacaatcccattgcacttatcacaacggagatgcgcatacttcaccagatgagctcactaggaaacgtgtcctgtcagtaatcacagagcctattctaccctttgagagataa

SEQ ID NO: 2 - protein, 595 aa, Populus nigra
MATELLCLHRPISLTHKLFRNPLPKVIQATPLTLKLRCSVSTENVSFTETETETRRSANYEPNSWDYDYLLSSDTDESIEVYKDKAKKLEAEVRREINNEKAEFLTLPELIDNVQRLGLGYRFESDIRRALDRFVSSGGFDAVTKTSLHATALSFRLLRQHGFEVSQEAFSGFKDQNGNFLKNLKEDIKAILSLYEASFLALEGENILDEAKVFAISHLKELSEEKIGKDLAEQVNHALELPLHRRTQRLEAVWSIEAYRKKEDADQVLLELAILDYNMIQSVYQRDLRETSRWWRRVGLATKLHFARDRLIESFYWAVGVAFEPQYSDCRNSVAKMFSFVTIIDDIYDVYGTLDELELFTDAVERWDVNAIDDLPDYMKLCFLALYNTINEIAYDNLKDKGENILPYLTKAWADLCNAFLQEAKWLYNKSTPTFDEYFGNAWKSSSGPLQLVFAYFAVVQNIKKEEIDNLQKYHDIISRPSHIFRLCNDLASASAEIARGETANSVSCYMRTKGISEELATESVMNLIDETWKKMNKEKLGGSLFAKPFVETAINLARQSHCTYHNGDAHTSPDELTRKRVLSVITEPILPFER

SEQ ID NO: 3 - DNA, 59 bp, Artificial
  oligonucleotide primer for PCR
ggccgcggatccagaatttaaaaggagggattaaaatggcaactgaattattgtgcttg

SEQ ID NO: 4 - DNA, 84 bp, Artificial
  oligonucleotide primer for PCR
ccgcgccggatccgacattaaaaaaataagagttaccatttaaggtaactcttatttttattatctctcaaagggtagaatagg

SEQ ID NO: 5 - DNA, 32 bp, Artificial
  oligonucleotide linker
gatcgctgcaggtttaaacggatccactaccg

SEQ ID NO: 6 - DNA, 32 bp, Artificial
  oligonucleotide linker
aattcggtagtggatccgtttaaacctgcagc

SEQ ID NO: 7 - DNA, 131 bp, Artificial
  oligonucleotide linker
gtttttaacaaaatatattgataaaaataataatagtgggtataattaagttgttagagaaaacgtataaattagggataaactatggaacttatgaaatagattgaaatggtttatctgttaccccgtag

SEQ ID NO: 8 - DNA, 139 bp, Artificial
  oligonucleotide linker
gatcctacggggtaacagataaaccatttcaatctatttcataagttccatagtttatccctaatttatacgttttctctaacaacttaattatacccactattattatttttatcaatatattttgttaaaaactgca

SEQ ID NO: 9 - DNA, 6441 bp, Streptomyces griseolosporeus
gttgactcttccgacctcggtggaggagggatcgaaggcccaccgggctcgcgccgtcggcaccggtcgcgctcatgccaaggccattctgctgggagagcacgcggtcgtgtacggaaccccggcgctcgcgatgcccattccccaactcgcggtcacggcaagcgccggctggtccggccgatccgccgagagccggggcggtccgaccttcaccatgaccgggtcggcttcccgcgcggtcacggcacaggccttggacggtctgcgacgtctgaccgcctcggtcaaggcgcacacgggagtgaccgacggacaacacctcgacgtcagcctcgacggggcgattccgcccggccgcgggctcggctccagcgccgcgaacgcacgagcgatcatcctcgccctggccgacctcttcggccgggagctgaccgagggcgaggtgttcgacctggtgcaggaggccgagaacctgacgcacggccgggccagcggcgtcgacgccgtgaccgtcggcgccaccgccccgctcctcttccgggcgggcacggcacaggcgctggacatcggctgcgacgcactgttcgtcgtcgcggacagcggaaccgcagggagcaccaaggaggcgatcgagctgcttcgcgccggattccgggccggggccggaaaggaggaacggttcatgcaccgtgccgcgcacctcgtcgacgatgccagggcctccctcgccgagggcgaacccgaggcgttcggatcgtgcctgaccgagtatcacggcctgctgcgcggggcgggtctgagcaccgaccggatcgatgcactggtggatgccgcgctgcaggccgacagcctgggcgccaagatcaccggtggcggtctgggcggttgtgttctcgcgatgtcccgcccggagcgggccgaggaagtggcccggcagctgcacgccgccggcgccgtacgcacgtgggccgtacagctgaggaggtccactcatgagcgctgaacagccgtcaaccctgctgtccgcgccgcgacggacaccgcgacagccgttgcccagccgaacatcgcgctgatcaagtactggggcaagaaggacgagcacctggtcctgccccgtaccgacagcctgtcgatgactctggacatcttcccgacgaccacccgggtccagctcgcgcccggcgccgggcaggacacggtggccttcaacggcgagcccgcgacgggagaggccgagcggcgcatcaccgcattcctccggctggtgcgggagcggtcggggcgcaccgaacgggcccgcgtcgagacggagaacaccgtccccaccggggccggcctggcctcgtcggccagcggtttcgctgccctcgccgtcgccgccgccgcggcgtacgggctcggtctcgacgcgcggggcctgtcccggctggcccgacgcggctccgggtcggcctcccggtcgatcttcgacgggttcgccgtgtggcacgccggccacgccggcggcactcccgaggaggccgatctcggctcgtacgccgaaccggtgccggccgtggacctggagccggcgctggtggtcgcggtggtcagcgccgcccccaaggcggtgtccagccgggaggccatgcggaggaccgtggacacctcaccgctgtacgagccgtgggcggtgtccagccgggccgacctggcggacatcggagccgcgctcgcccgcggcaacctgccggcggtgggcgagatcgcggagcgcaacgccctcggcatgcacgccaccatgctggccgcacgccccgccgtgcgctacctgtcaccggcctcgctcgccgtgctcgacggcgttctgcagttgcggcgggacggcgtgccggcctacgcgacgatggacgccggtcccaacgtgaaggtgctctgcccgcgttcggacgccgagcgggtcgcggaagccctgcgcgccgccgcgccggtcggagcggtgcacatcgccggtccggggcggggtgcccgcctggtggcggaggaatgccggtgaccggcccgcgcgcggtgacccggcgcgccccgggcaagctcttcgtcgcgggtgaatacgcggtggtggaaccgggcaaccgggcgatcctggtggcagtcgaccggtacgtcaccgtcaccgtgtccgacggcgccgcacccggtgtcgtcgtctcctccgacatcggagccggcccggtgcaccacccgtggcaggacgggcggctgacaggcggtacgggcacacctcatgtggtggcggcggtcgagaccgtggcccgcctcctggccgaacgcggccggtccgtcccgccgttggggtggtcgatcagcagcacgctgcacgaggacggccggaagttcggactgggctccagcggcgcggtgacggtggcgacggtcagtgccgtcgcagcccattgcggactggaactcaccgccgaagaacgcttccggacggcgctgatcgcctccgcccgcatcgaccccaggggatccggcggagacatcgccaccagcacctggggcggctggatcgcctaccgggcgcccgaccgggacgccgtactcgacttgacccgccgtcagggggtcgacgaggcactccgggcgccgtggccgggcttctccgtacgactgtcgccgccccggaacctctgcctcgaggtcggctggaccggcaaccccgtgtccaccacgtccctcctgacggacctgcatcggcgcacctggcggggcagccccgcgtaccggaggtacgtcggggcgaccggcgagctcgtggacgccgcagtcatcgcgctggaggacggcgacaccgagggcctgttgcggcaggtccggcgggcccgtcacgagatggtccgcctcgacgacgaggtcggcctcggcatcttcacccccgaactgacggccctctgcgccatcgccgaacgcgccggcgcggccaagccctcgggggccgggggcggcgactgcggcatcgcgctgctggacgccgaggcccgctacgaccgctcaccgttgcaccggcaatgggccgcggccggggtgctgccgctactggtgtcgcctgccacggaaggagtcgaggaatgagcagtgcccagcgcaaggacgaccatgtccggctcgccacggagcagcagcgcgcgcacagcggacgcaaccagttcgacgacgtgtcgttcgtccaccacgccctcgccggaatcgaccggccggacgtccgcctggccacgacgttcgccggcatcacctggcgactgccgctgtacatcaacgcgatgacgggcggcagcgccaagaccggcgccatcaaccgggacctggccgtcgccgccagggagaccggcgccgccatcgcgtccgggtccatgcacgcctttttcagggacccctcctgcgcggacaccttccgcgtgctgcgcaccgagaaccccgacggtttcgtgatggcgaacgtcaacgcgaccgcgtccgtcgacaacgcccgccgggccgtcgacctgatcgaggcgaacgccctgcagatccacctgaacacggcgcaggagacgcccatgccggagggcgaccggtcgttcgggtcgtggccggcccagatcgcgaagatcacggcggccgtcgacgtcccggtgatcgtcaaggaggtcggcaacgggctcagcaggcagaccctcctggcgctgccggatctgggggtccgggtcgccgacgtcagcggccgcggcggcaccgacttcgcccgtatcgagaacagccggcgccccctgggcgactacgccttcctgcacggctgggggcagtccaccccggcctgtctgctggacgctcaggacgtcggcttccccctgctggcctccggtgggatccgcaacccgctcgacgtcgcccgggcgctcgcgctcggcgccggcgccgtgggctcctcgggcgtattcctgcgcacgctgatcgacgggggcgtatccgccctggtcgcacagatctccacctggctggaccagctcgccgcgctgcagaccatgctcggtgcgcggacccccgccgacctcacccgctgcgacgtgctgatccacggcccgctccggtccttctgcacggaccggggcatagacatcgggcggttcgcccggcgcagcagctccgccgacatccgttccgagatgacaggaagcacacgatgaccgaagcgcacgccaccgccggcgtcccgatgcggtgggtggggcccgtccgcatctcgggaaacgtcgccaccatcgaaacccaggtgccgctggccacgtacgagtctccgctctggccttcggtgggccgcggcgcgaaggtgtcccggctgaccgagaagggcatcgtcgccacgctcgtcgacgagcgcatgacccgttccgtgctcgtcgaggcgaccgacgcgctcaccgcgctctccgcggcacggaccatcgaggcccgcatcgacgagctgcgcgagctggtgcgcggctgcagccggttcgcccagctgatcggcatccggcacgagatcaccggaaacctgctgttcgtccggttcgagttcagcaccggtgacgcctccgggcacaacatggcgaccctggcttccgacgtgctcctccagcatctgctggaaacggttcccggcatctcctacgggtcgatctccgggaactactgcacggacaagaaggccaccgccatcaacggcatcctgggccgcggcaagaacgtcgtcaccgagctgctcgtgccgcgtgacgtggtggccgacgtcctgaacaccaccgccgcgaagatcgccgagctgaacctccgcaagaacctgctcgggacacttctcgcaggcggcatccggtcggcgaacgcccactacgcgaacatgctgctcgcgttctacctggcgaccggtcaggacgcggcgaacatcgtcgagggctcccagggcgtcgtcacggccgaggaccgcgacggcgacctctacttagcctgcacactgccgaacctcatcgtcggcacggttggcaacggcaagggcctgggcttcgtggagaccaacctgaaccggctcggctgccgtgcggaccgcgagcccggcgagaacgcccgccggctcgccgtcatcgcggcggccacggtgctctgcggggagctgtcgctgctcgcggcgcagaccaaccccggcgaactgatgcgtgcgcatgtccaactggaacgaggccacacgaccgcgaaggctggtgtctagagcatgcccctcgccataggcatccatgatctgtcgttcgccaccggcgagttcggctgccgcacaccgccctcgccgctcacaacggaaccgagatcggcaagtaccacgcgggcatcggccaggagtcgatgagcgtcccggccgccgacgaggacatcgtgaccctggccgcgacggctgccgcaccgatcgtcgcccggcacggcagcgaccggatccgcacggtcgtgctcgcgaccgaatcgtcgatcgaccaggcgaagtcggccggtgtgtacgtccactccctgctcggactgccgtcggccacccgcgtcgtggagctgaagcaggcctgttacggggccacggccggcctgcagttcgccatcggtctggtgcagcgcgaccccgcccagcaggttctcgtcatcgccagtgacgtctccaagtacgacctggacagccccggtgaggcgacgcagggcgccgccgcggtcgccatgctcgtaggcgccgatccggggctggtgcggatcgaggatccgtcgggcctgttcaccgtcgacgtcatggacttctggcggccgaactaccgcaccacggctctggtcgacggccaggaatccatcggcgcctacctccaggcggtggagggggcctggaaggactactcggagcggggcggccactccctggagcagttcgccgcgttctgctaccaccagccgttcaccaagatggctcacaaggcccaccggcacctgctgaactactgcagccacgacatccaccacgacgacgtcacgcgtgccgtcggccggaccaccgcctacaacagggtgatcgggaacagctacaccgcgtccgtctacctgggcctcgccgcgctcctcgaccaggccgacgacctgaccggtgagcgcatcggattcctcagctacggttccggcagcgtcgccgagttcttcggcgggatcgtcgtcgccggataccgggaccggctgcggacggcggcgaacatcgaggccgtctcccggcgacggcccatcgactacgccggctaccgcgagctgcacgagtgggccttccccgcccgacggggagcccactccaccccgcagcagaccacgggaccgttccggctgtccggtatcagcggccacaagcgcctctaccgagcgtgctga

SEQ ID NO: 10 - DNA, 62 bp, Artificial
  oligonucleotide primer for PCR
cgggtaccaattttgttaataattcagggagggattctaaatgactcttccgacctcggtgg

SEQ ID NO: 11 - DNA, 71 bp, Artificial
  oligonucleotide primer for PCR
aggtaccattaaaaaaataagagttaccatttaaggtaactcttatttttatcagcacgctcggtagaggc

SEQ ID NO: 12 - DNA, 39 bp, Artificial
  oligonucleotide primer for PCR
tggtaccttattcttttatctctcaaagggtagaatagg

SEQ ID NO: 13 - DNA, 15 bp, Artificial
  oligonucleotide linker
gatccggtacctttg

SEQ ID NO: 14 - DNA, 15 bp, Artificial
  oligonucleotide linker
aattcaaaggtaccg

SEQ ID NO: 15 - DNA, 2620 bp, Artificial
  Designed polynucleotide containing Isopentenyl diphosphate isomer ase gene and isoprene synthase gene
ctgcagtttttaacaaaatatattgataaaaataataatagtgggtataattaagttgttagagaaaacgtataaattagggataaactatggaacttatgaaatagattgaaatggtttatctgttaccccgtaggatcgagaatttaaaaggagggattaaaatgcaaactgaacatgttattttattgaatgcacagggagttcctactggtactctggaaaagtatgccgcacatacagcagacacccgcttacatctcgctttctccagttggctgtttaatgccaaaggacaattattagttaccagaagagcactgagcaaaaaagcatggcctggcgtgtggactaactctgtttgtgggcatccacaactgggagaaagcaacgaagacgcagtgatcagaagatgtcgttatgagcttggcgtggaaattactcctcctgaatctatctatcctgactttagatacagagccaccgatcctagtggcattgtggaaaatgaagtgtgtcctgtatttgccgcaagaaccactagtgcattacagatcaatgatgatgaagtgatggattatcaatggtgtgatttagcagatgtattacatggtattgatgccactccttgggctttcagtccttggatggtgatgcaggcaacaaatagagaagccagaaaaagattatctgcatttacccagcttaaataattaataattaattcgaacagaaaaaataagtatttatataacggttaattgtaaggagggttttttatggcaactgaattattgtgtttgcatagaccaatctcactgacacataaattgttcagaaatcctttgcctaaagttatccaggccactcctttaactttgaaacttagatgttctgtaagcacagaaaacgtaagcttcacagaaacagaaacagaaaccagaaggtctgccaattatgaaccaaatagctgggattatgattatttgctgtcttctgacactgacgaatctattgaagtatacaaagacaaggccaaaaagctggaggctgaggtgagaagagagattaacaatgaaaaggcagagtttttgactctgcctgaactgatagataatgttcaaaggttaggattaggttacagattcgagagtgacataaggagagcccttgatagatttgtttcttcaggaggatttgatgctgttacaaaaactagccttcatgctactgctcttagcttcaggcttctcagacagcatggctttgaggtatctcaagaagctttcagcggattcaaggatcaaaatggcaatttcttgaaaaaccttaaggaggacatcaaggcaatactaagcctatatgaagcttcatttcttgccttagaaggagaaaatatcttggatgaggccaaggtgtttgcaatatcacatctaaaagagcttagcgaagaaaagattggaaaagacctggccgaacaggtgaatcatgcattggagcttccattgcatagaaggacacaaagactagaagctgtttggagcattgaagcatacagaaaaaaggaagatgcagatcaagtactgctagaacttgctatattggactacaacatgattcaatcagtataccaaagagatcttagagagacatcaaggtggtggaggagagtgggtcttgcaacaaagttgcattttgctagagacaggttaattgaaagcttttactgggcagttggagttgcatttgaacctcaatacagtgattgtagaaattccgtagcaaaaatgttttcttttgtaacaatcattgatgatatctatgatgtttatggtactctggatgagttggagctatttacagatgctgttgagagatgggatgttaatgccatcgatgatcttcctgattatatgaagctttgtttcctagctctttataacactatcaatgagatagcttatgataatctgaaggacaagggggaaaacattcttccatacctaacaaaagcatgggcagatttatgtaatgcattcctacaagaagcaaaatggttgtacaataagtccacaccaacatttgatgaatatttcggaaatgcatggaaatcatcctcagggcctcttcaactagtttttgcctactttgccgttgttcaaaacatcaagaaagaggaaattgataacttacaaaagtatcatgatatcatcagtaggccttcccatatctttagactttgtaacgacttggcttcagcatctgctgagatagcaagaggtgaaaccgcaaattctgtatcatgttacatgagaacaaaaggcatttctgaggaacttgctactgaatccgtaatgaatttgatcgacgaaacctggaaaaagatgaacaaagaaaagcttggtggctctctgtttgcaaaaccttttgttgaaacagctattaaccttgcaagacaatcccattgtacttatcataacggagatgcacatacttcaccagatgagcttactaggaaaagagtactgtcagtaatcacagagcctattctaccttttgagagataataaaaataagagttaccttaaatggtaactcttatttttttaatgtcggatcc

SEQ ID NO: 16 - DNA, 549 bp, Escherichia coli
atgcaaacggaacacgtcattttattgaatgcacagggagttcccacgggtacgctggaaaagtatgccgcacacacggcagacacccgcttacatctcgcgttctccagttggctgtttaatgccaaaggacaattattagttacccgccgcgcactgagcaaaaaagcatggcctggcgtgtggactaactcggtttgtgggcacccacaactgggagaaagcaacgaagacgcagtgatccgccgttgccgttatgagcttggcgtggaaattacgcctcctgaatctatctatcctgactttcgctaccgcgccaccgatccgagtggcattgtggaaaatgaagtgtgtccggtatttgccgcacgcaccactagtgcgttacagatcaatgatgatgaagtgatggattatcaatggtgtgatttagcagatgtattacacggtattgatgccacgccgtgggcgttcagtccgtggatggtgatgcaggcgacaaatcgcgaagccagaaaacgattatctgcatttacccagcttaaataa

SEQ ID NO: 17 - DNA, 2545 bp, Artificial
  Designed polynucleotide containing Isopentenyl diphosphate isomer ase gene and isoprene synthase gene
atgacagcagataacaattctatgccacatggagcagtttcaagttatgcgaaattagttcagaaccaaactccagaagacatactagaggaatttccagaaatcatacccttacaacaaagaccaaatacaagaagttcggaaacatctaatgatgaatcaggtgaaacttgtttttcaggacatgatgaagaacagatcaaactcatgaacgagaattgtattgttcttgattgggacgataatgctataggtgctggtactaaaaaggtttgtcacttaatggaaaatatcgaaaagggattgttacacagagcatttagtgtatttatctttaatgaacaaggagaattactacttcaacaaagagctacagaaaagataacgtttcctgatttatggaccaatacttgttgtagtcatcctctatgtatagatgatgagttaggacttaaaggcaaattagacgacaaaatcaaaggtgctataacagcagctgtaagaaagttagatcatgagttaggaatacctgaagatgagactaaaactagaggaaaattccattttcttaaccgtatccattatatggcaccttctaatgaaccttggggtgaacatgaaatcgattatatcttgttctacaaaatcaatgctaaggaaaatcttactgtgaatcccaatgtaaatgaagtaagagattttaagtgggttagtcctaatgatctgaaaaccatgtttgcagatccttcctataaatttacaccttggtttaagattatatgcgagaattatctctttaattggtgggaacaattggatgatttgagtgaagttgagaatgacagacaaatacatcgaatgttatagtagtgataccgtttaaacaggaagaatcatagaggaggaatcaatggaagcgagacgcagtgccaattatgaaccaaatagctgggattatgattatcttctgagtagtgataccgatgaaagcattgaagtatataaagataaagccaaaaaattagaagcagaagtgagacgtgaaattaataatgaaaaagctgaatttctgacactgttagaacttattgataatgtgcagcgcctgggattaggctatagatttgaaagcgatattagaggcgcactggatcgttttgtgagttcaggtggatttgatgctgttacaaaaactagccttcatggaactgcgctgagttttcgccttctgagacagcacggctttgaagttagccaagaagcctttagtggttttaaagatcaaaatggaaattttctggaaaatcttaaagaagatattaaagcaatactttcactgtatgaagcaagttttctggcacttgaaggagaaaatatacttgatgaagctaaagtttttgcgatttcacatcttaaagaactgtctgaagaaaaaattggcaaagaactggctgaacaggttaatcatgcgctggaattaccgcttcaccgcagaacccaaagattagaagccgtttggtctattgaagcatatcgtaaaaaagaagatgccaatcaggtacttcttgaattagcaatacttgattataatatgattcagagcgtgtatcaacgtgatcttcgcgaaaccagtagatggtggcgtcgcgttggccttgctacgaaactgcattttgcgagagatcgtctgattgaaagcttttattgggccgtgggtgttgcatttgaaccacaatatagcgattgtcgtaatagtgttgcaaaaatgtttagttttgtaactataattgatgatatttatgatgtttatggtacacttgatgaactggaactttttactgatgctgtagaacgctgggatgtgaatgcgattaatgatctgccagattatatgaaactttgttttcttgccctgtataatacaattaatgaaattgcatatgataatcttaaagataaaggagaaaatatactgccttatttaactaaagcatgggctgatttatgcaatgcttttcttcaggaagcgaaatggctgtataataaatcaacccctacgtttgatgattattttggcaatgcttggaaatctagcagtggtccgttacagcttgtttttgcttattttgcggttgtacaaaatattaaaaaagaagaaattgaaaatctgcaaaaatatcatgatactatttcacgtccttctcacatatttcgcttatgtaatgatcttgcgtcagcaagtgcagaaattgcccgcggtgaaaccgcaaatagcgtaagttgctatatgagaacaaaaggaatttcagaagaacttgcaactgaatctgtgatgaatctgattgatgaaacctggaagaaaatgaataaagaaaaattaggcggttctctgtttgctaaaccatttgtagaaacggctataaatcttgcgcgtcagtcacattgcacctatcacaatggagatgcgcatacgtctccggatgaacttaccagaaaaagagtgctgagtgtgattaccgaaccgatactgccatttgaacgctaa

SEQ ID NO: 18 - DNA, 9237 bp, Artificial
  Escherichia coli/Clostridium shuttle vector pSCi01
tcgaccttcaggtttgtctgtaactaaaaacaagtatttaagcaaaaacatcgtagaaatacggtgttttttgttaccctaagtttcagggccccctgcttcggggtcattatagcgattttttcggtatatccatcctttttcgcacgatatacaggattttgccaaagggttcgtgtagactttccttggtgtatccaacggcgtcagccgggcaggataggtgaagtaggcccacccgcgagcgggtgttccttcttcactgtcccttattcgcacctggcggtgctcaacgggaatcctgctctgcgaggctggccggctaccgccggcgtaacagatgagggcaagcggatggctgatgaaaccaagccaaccaggaagggcagcccacctatcaaggtgtactgccttccagacgaacgaagagcgattgaggaaaaggcggcggcggccggcatgagcctgtcggcctacctgctggccgtcggccagggctacaaaatcacgggcgtcgtggactatgagcacgtccgcgagctggcccgcatcaatggcgacctgggccgcctgggcggcctgctgaaactctggctcaccgacgacccgcgcacggcgcggttcggtgatgccacgatcctcgccctgctggcgaagatcgaagagaagcaggacgagcttggcaaggtcatgatgggcgtggtccgcccgagggcagagccatgacttttttagccgctaaaacggccggggggtgcgcgtgattgccaagcacgtccccatgcgctccatcaagaagagcgacttcgcggagctggtgaagtacatcaccgacgagcaaggcaagaccgatcgggccccctaaacgagtgactcgagaacatgtgagcaaaaggccagcaaaaggccaggaaccgtaaaaaggccgcgttgctggcgtttttccataggctccgcccccctgacgagcatcacaaaaatcgacgctcaagtcagaggtggcgaaacccgacaggactataaagataccaggcgtttccccctggaagctccctcgtgcgctctcctgttccgaccctgccgcttaccggatacctgtccgcctttctcccttcgggaagcgtggcgctttctcatagctcacgctgtaggtatctcagttcggtgtaggtcgttcgctccaagctgggctgtgtgcacgaaccccccgttcagcccgaccgctgcgccttatccggtaactatcgtcttgagtccaacccggtaagacacgacttatcgccactggcagcagccactggtaacaggattagcagagcgaggtatgtaggcggtgctacagagttcttgaagtggtggcctaactacggctacactagaagaacagtatttggtatctgcgctctgctgaagccagttaccttcggaaaaagagttggtagctcttgatccggcaaacaaaccaccgctggtagcggtggtttttttgtttgcaagcagcagattacgcgcagaaaaaaaggatctcaagaagatcctttgatcttttctacggggtctgacgctcagtggaacgaaaactcacgttaagggattttggtcatgagattatcaaaaaggatcttcacctagatccttttaaattaaaaatgaagttttaaatcaatctaaagtatatatgagtaaacttggtctgacagcctgcaggtaatacgactcactatagggataacttaaatttatattttttactttataatatataattgattatagaatccaaattagataggaggaccaggtaaatggagaataattttattgtcaacgaaaacgagaaaagggttttaaagcagatatttaacaactccaatatcagtagaactcaaatttccaagaatttagaactgaataaagcaacaatttcgaacattcttaacaatctaaagcataaaagtttggtaaatgaagttggtgaaggaaattctactaaaagtggtggaagaaaacctatacttctcgaaattaatcaaaagtatgggtattatataagcatggatttgacatatgattctgttgagttaatgtataactattttgatgctacaattctcaaacaagatagttatgaactgaatgataagaatgtaagtagcatattacagatactcaaatctaacataaatgttagcgaaaaatacgacacattatacggtttattagggataagtatatccatacatgggattgtagatgatgaacaaaacatcattaatctaccatttcacaagaatgaaaaaagaacgtttactgatgaacttaagtctttcactaatgtaccagtggttattgaaaatgaggcaaatttaagtgcattatacgagaaaagtttatacatcaattcgaatattaacaacttgatcacattgtctatacataaaggtataggagctggcatcataatcaataagaaactctatagaggtagtaatggagaagctggagaaataggaaagactcttgttttagagtctatcaataacaatgataacaagtactataaaatagaggatatttgtagtcaagacgctttgatacaaaagattaataacagattaggagttacacttacatttaccgaactaatacagtattataacgaaggaaatagtattgtagctcatgaaatcaaacagtttatcaacaaaatgactgtcttaatacacaatcttaatactcagtttaatccagatgcaatatacatcaattgtcccttgattaatgaacttcctaatattctaaacgaaatcaaagaacaattctcttgtttttcacaaggaagtcctatacaattgcatttaaccactaatgttaaacaagctacattattaggtggaacattagcaattatgcagaaaacccttaacataaacaatatccaaatgaatattaaatagttacagcagtctgagttataaaatagatatctcggaccgtctattcttccttatttgagtgggtaccaatgaaatctttcgagctaaatcgatttctggcccactcttttttattttttagtaagcgtttacaaaaaatgaacaatgtgctatattacctctaaagttagtttgtttattaaattaaccaactaaaatgtcgggatccaattaggaggaatctgcgatggaaaagaaggaatttagagttttaataaagtattgttttcttaaaggaaagaatacagtagaagctaagacttggttagataatgaatttccagattctgctcctggtaaaagtacaattatagattggtatgcaaaatttaaaagaggagaaatgtcaacagaagatggagaaagatctggtagaccaaaagaagttgtaactgatgaaaatataaagaagatacataaaatgatattaaatgatagaaagatgaagttaatagaaatagcagaagctttaaaaatatctaaagaaagagttggacatataatacatcaatatttagatatgagaaaattatgtgcaaaatgggttccaagagaattaacttttgatcaaaagcaaagaagagtagatgatagtaagagatgtttacaattattaacaagaaatactccagaatttttcagaagatatgtaacaatggatgaaacttggttacatcattatacacctgaaagtaatagacaatcagcagaatggacagctactggagaaccatcacctaaaagaggaaagactcaaaagagtgctggaaaggttatggcatcagtattttgggatgctcatggtataatatttatagattatttagaaaaaggaaaaacaataaattctgattattatatggcattattagaaagattaaaagttgaaatagcagctaaaagaccacatatgaagaagaaaaaagtattatttcatcaagataatgctccttgtcataagtcattaagaactatggcaaagatacatgaattaggttttgaattattaccacatccaccttattcaccagatttagctccttctgatttctttttatttagtgatttaaagagaatgttagcaggaaagaagtttggttgtaatgaagaagttatagcagaaacagaagcttattttgaagcaaaacctaaggaatattatcaaaatggaataaagaagttagaaggtagatataatagatgtatagcattagaaggaaattatgtagaataagaattccttaattaaggagctcgataaaaataagaagcctgcatttgcaggcttcttatttttatggtcatagctgtttcctggcgcgccgccattatttttttgaacaattgacaattcatttcttattttttattaagtgatagtcaaaaggcataacagtgctgaatagaaagaaatttacagaaaagaaaattatagaatttagtatgattaattatactcatttatgaatgtttaattgaatacaaaaaaaaatacttgttatgtattcaattacgggttaaaatatagacaagttgaaaaatttaataaaaaaataagtcctcagctcttatatattaagctaccaacttagtatataagccaaaacttaaatgtgctaccaacacatcaagccgttagagaactctatctatagcaatatttcaaatgtaccgacatacaagagaaacattaactatatatattcaatttatgagattatcttaacagatataaatgtaaattgcaataagtaagatttagaagtttatagcctttgtgtattggaagcagtacgcaaaggcttttttatttgataaaaattagaagtatatttattttttcataattaatttatgaaaatgaaagggggtgagcaaagtgacagaggaaagcagtatcttatcaaataacaaggtattagcaatatcattattgactttagcagtaaacattatgacttttatagtgcttgtagctaagtagtacgaaagggggagctttaaaaagctccttggaatacatagaattcataaattaatttatgaaaagaagggcgtatatgaaaacttgtaaaaattgcaaagagtttattaaagatactgaaatatgcaaaatacattcgttgatgattcatgataaaacagtagcaacctattgcagtaaatacaatgagtcaagatgtttacataaagggaaagtccaatgtattaattgttcaaagatgaaccgatatggatggtgtgccataaaaatgagatgttttacagaggaagaacagaaaaaagaacgtacatgcattaaatattatgcaaggagctttaaaaaagctcatgtaaagaagagtaaaaagaaaaaataatttatttattaatttaatattgagagtgccgacacagtatgcactaaaaaatatatctgtggtgtagtgagccgatacaaaaggatagtcactcgcattttcataatacatcttatgttatgattatgtgtcggtgggacttcacgacgaaaacccacaataaaaaaagagttcggggtagggttaagcatagttgaggcaactaaacaatcaagctaggatatgcagtagcagaccgtaaggtcgttgtttaggtgtgttgtaatacatacgctattaagatgtaaaaatacggataccaatgaagggaaaagtataatttttggatgtagtttgtttgttcatctatgggcaaactacgtccaaagccgtttccaaatctgctaaaaagtatatcctttctaaaatcaaagtcaagtatgaaatcataaataaagtttaattttgaagttattatgatattatgtttttctattaaaataaattaagtatatagaatagtttaataatagtatatacttaatgtgataagtgtctgacagtgtcacagaaaggatgattgttatggattataagcggccggccagtgggcaagttgaaaaattcacaaaaatgtggtataatatctttgttcattagagcgataaacttgaatttgagagggaacttagatggtatttgaaaaaattgataaaaatagttggaacagaaaagagtattttgaccactactttgcaagtgtaccttgtacctacagcatgaccgttaaagtggatatcacacaaataaaggaaaagggaatgaaactatatcctgcaatgctttattatattgcaatgattgtaaaccgccattcagagtttaggacggcaatcaatcaagatggtgaattggggatatatgatgagatgataccaagctatacaatatttcacaatgatactgaaacattttccagcctttggactgagtgtaagtctgactttaaatcatttttagcagattatgaaagtgatacgcaacggtatggaaacaatcatagaatggaaggaaagccaaatgctccggaaaacatttttaatgtatctatgataccgtggtcaaccttcgatggctttaatctgaatttgcagaaaggatatgattatttgattcctatttttactatggggaaatattataaagaagataacaaaattatacttcctttggcaattcaagttcatcacgcagtatgtgacggatttcacatttgccgttttgtaaacgaattgcaggaattgataaatagttaacttcaggtttgtctgtaactaaaaacaagtatttaagcaaaaacatcgtagaaatacggtgttttttgttaccctaagtttaaacccagagcctacgagttccgaactagacaggttggctgataagtccccggtctggcgcgacatcataacggttctggcaaatagtgacttctgaaatgagcataaaaataagaagcctgcaaatgcaggcttcttatttttatggggaattgttatccgctcacaattcccctatagtgagtcgtattaatttcgccatggtacgtaaggcctatttaaatcacgtgcggccgcatgtacagcgacgtcactagtctaagttccctcctaaaattcaagtttatcgctctaatgaacaaagatattatactctatcaatgatagagtttcaaactctatcaatgatagagtgaatccgttagcgaggttgagttatcgagattttcaggagcgggtgctagctgagcccgcggaacagctgtcccgggagaagttcctatactttctagagaataggaacttcggaataggaacttcttagggtaacaaaaaacaccgtatttctacgatgtttttgcttaaatacttgtttttagttacagacaaacctgaaggaattcctaagatccactttcacacttaagctgtttctctagtccgcaaattattaactccaatccaaagagaaacgcaggttcagctccttgatgatcaaacagttctatagcttgtcgtaataaaggtggcatactatctgtagtaggagtttctctctcttcttttgcaacttgatgttcttgatcttccaaaacacaacctaacgtgaaatgacctacagctgaaagagcatataatgcgttctctaatgagaatccttgttgacatagaaatgccaactgattttcaagtgtctcatactgcttttctgtaggtctagttcctaagtgaactttagccccatctctatgggatagtaaagcacatctgaaacttttcgcgttattcctcaaaaagtcttgccaactttcaccttctaatggacaaaagtgtgtatgatgtctgtctaacatttcgattgctaatgcatctaagagtgctcttttgtttttgacatgccagtacaatgttggttgttcaactccaagtttctgagctaatttcctggtagttagaccttcaattccaacttcattaaggagttctaatgcggaatttatcactttagacttatcgagtctactcattctaactaacctcctaacaacttaattatacccactattattatttttatcaatatatgcctgcagcgaccaaaagtataaaacctttaagaactttcttttttcttgtaaaaaaagaaactagataaatctctcatatcttttattcaataatcgcatcagattgcagtataaatttaacgatcactcatcatgttcatatttatcagagctcgtgctataattatactaattttataaggaggaaaaaataaagagggttataatgaacgagaaaaatataaaacacagtcaaaactttattacttcaaaacataatatagataaaataatgacaaatataagattaaatgaacatgataatatctttgaaatcggctcaggaaaagggcattttacccttgaattagtacagaggtgtaatttcgtaactgccattgaaatagaccataaattatgcaaaactacagaaaataaacttgttgatcacgataatttccaagttttaaacaaggatatattgcagtttaaatttcctaaaaaccaatcctataaaatatttggtaatataccttataacataagtacggatataatacgcaaaattgtttttgatagtatagctgatgagatttatttaatcgtggaatacgggtttgctaaaagattattaaatacaaaacgctcattggcattatttttaatggcagaagttgatatttctatattaagtatggttccaagagaatattttcatcctaaacctaaagtgaatagctcacttatcagattaaatagaaaaaaatcaagaatatcacacaaagataaacagaagtataattatttcgttatgaaatgggttaacaaagaatacaagaaaatatttacaaaaaatcaatttaacaattccttaaaacatgcaggaattgacgatttaaacaatattagctttgaacaattcttatctcttttcaatagctataaattatttaataagtaagttaagggatgcataaactgcatcccttaacttgtttttcgtgtacctattttttgtgaatcgattatgtcttttgcgcattcacttcttttctatataaatatgagcgaagcgaataagcgtcggaaaagcagcaaaaagtttcctttttgctgttggagcatgggggttcagggggtgcagtatcgaagttcctatactttctagagaataggaacttcggaataggaacttcccgggaatgtagaccggggacttatcagccaacctgttagatggcccgcacgatcaaggcgcgccaggaaacagctatgaccg

SEQ ID NO: 19 - DNA, 2545 bp, Artificial; identical to SEQ ID NO: 17
  Expression vector pSCi::idi-isps

SEQ ID NO: 20 - DNA, 9818 bp, Artificial
  Isoprene synthase gene cluster
atttaaatactatcaagagaagaataaagaaggaggtttaaaaatgaaaaattgtgtaattgtgagtgctgtaagaacagcaataggaagctttaatggatcattggctagtacatctgcaattgatcttggtgcaactgtaataaaggctgctattgaaagagcaaaaattgattcacaacatgttgacgaagtaataatgggaaacgtattacaagcaggacttggacaaaatccagcaagacaggcacttttgaaaagtggattagctgaaactgtatgtggattcactgttaataaggtttgtggttctggacttaaatctgtagcacttgcagctcaagctatacaagctggacaagctcagtcaatagttgctggtggcatggaaaatatgtcattggcaccttatcttcttgatgcaaaagcaagatcaggatatagattgggtgatggacaagtgtatgatgtaatattaagagacggattaatgtgcgcaactcatggataccatatgggtataacagctgaaaatgtagcaaaagagtatggaataacaagagagatgcaagatgagttagctcttcattctcagagaaaagctgctgctgctattgaatctggtgcttttactgcagaaatagtaccagttaatgtagtgactaggaaaaagacttttgtttttagccaagatgaatttcctaaagcaaacagtacagcagaagcattaggcgcattaaggcctgcttttgataaagctggtacagttacagctggaaatgctagtggaattaatgacggtgctgctgcattggttataatggaagaaagtgctgctttagctgcaggacttactcctttagcaaggattaaaagctatgcatctggtggcgtaccaccagcattaatgggtatgggtcctgttccagcaacacagaaggcattgcaattagcaggattacagttagctgatattgatttgattgaggcaaatgaagcttttgctgctcagtttttagcagtaggtaagaatcttggatttgatagtgaaaaagtaaacgttaatggtggcgcaatagcacttggacatcctattggtgcatcaggtgctagaatacttgtgacattattacacgctatgcaagctagagataaaactttaggtcttgcaactttatgtattggcggtggccagggtatagcaatggttatagaaagattaaattaaggatcccaataaacagggattaacatataggaggtaaaataatgacaataggcatagacaaaatatcatttttcgtacctccttattatatagatatgactgcattagctgaggcaagaaatgttgatcctggtaaattccacattggaataggacaagatcaaatggcagttaatccaatttctcaagatatagttacatttgctgctaacgcagctgaggcaattcttactaaagaagacaaagaagcaattgatatggtaatagtaggtactgaatctagtatagatgagtctaaggctgcagctgttgttttacacagattaatgggtattcaaccttttgctagaagctttgaaattaaagaagcttgttatggcgctacagcaggtcttcaattggctaaaaatcatgtagctcttcatcctgataagaaagtattagtagtggcagcagacatagcaaaatatggattgaattctggtggtgaacctactcaaggcgctggtgcagtagcaatgttagtggcatcagaacctagaattcttgctttaaaagaagataacgttatgttgactcaggacatatatgatttttggagaccaacaggtcatccatatccaatggttgatggaccattgagtaatgagacttatattcagagctttgctcaagtttgggatgagcataagaaaagaacaggacttgattttgctgattacgatgcattagcatttcatattccatacactaaaatgggtaaaaaggctttattagcaaagataagtgaccaaactgaggcagaacaagaaagaatattagctaggtacgaagaaagtattatttattcaagaagagttggaaatttatacactggtagcctttatttgggtttaatatctttacttgagaatgctacaacacttacagctggtaatcaaataggattgtttagttatggctctggtgcagtagcagaatttttcactggcgaacttgtagcaggatatcagaatcacttacaaaaagaaactcatttagcattacttgacaatagaacagagcttagtattgcagaatatgaggctatgtttgctgagacacttgatacagatatagatcagacacttgaagacgaattgaaatactcaatatcagctataaacaatactgtaaggtcatatagaaattaaccatggtggaatacaatagagacatataaggaggacaaaaaatggttgcagattcaagattacctaattttagagctcttacaccagctcagagaagagatttcttagctgatgcatgtggattgtcagatgcagaaagggcattacttgctgctcctggtgctttaccattagcattagcagacggtatgattgaaaatgtttttggatcttttgaattaccacttggcgttgctggaaattttagagttaacggaagagatgttcttgttccaatggctgtagaagaaccttcagtggtagcagcagcatcttatatggctaagcttgcaagagaagacggcggttttcaaacttcttctactttacctttaatgagagcacaggtacaagtattaggtgtgacagatcctcatggcgctaggttagcagttcttcaagctagagctcaaataatagaaagggcaaattcaagagataaagttttaataggacttggtggtggctgcaaagatatagaagtacacgtatttccagatactcctagaggtcctatgcttgtagttcatttaatagttgacgtaagagacgctatgggtgctaatacagttaatacaatggctgaaagtgttgcacctttagtggaaaagattactggcggtagtgtaagattaagaattctttcaaatcttgcagatcttagattagctagggctagagtaagattgacaccacagacattggctacacaagatagaagtggtgaagagataatagaaggtgtacttgacgcatatacatttgctgctattgatccatatagggctgctactcataataaaggtataatgaacggtattgatccagttattgtagctactggaaacgattggagagcagtggaagcaggtgcacatgcttatgcaagtagaagcggaagttacactagcttgactagatgggaaaaagatgctggcggtgctcttgtaggatctatagaacttccaatgccagtaggacttgtgggtggtgcaactaaaactcatcctttggcaaggttggcacttaaaataatggatttgcaaagtgcacaacaacttggtgagatagctgctgcagttggattggcacagaatcttggtgcattaagggctttagcaactgaaggtatacaaagaggccatatggctttgcacgctagaaatattgctttagtagctggtgctacaggtgatgaagttgatgctgttgctaggcagcttgctgctgaacatgacgttagaacagatagggcacttgaagttttagctgcacttagagcaagagcttaagttcaaacactatcataacacacaatagaaaggaggataaaaaatggtttcatgtagcgcaccaggtaagatatatttatttggtgaacatgctgtagtatatggcgaaacagctatagcatgcgctgtagaattaaggactagggtaagagcagaacttaacgattcaataacaatacaatcacagattggtagaacaggacttgattttgaaaagcacccatatgtatctgctgtaattgaaaagatgagaaaatcaatacctataaatggtgtattcttgactgttgatagtgacatacctgttggatctggacttggatcttcagcagcagttactattgcttctattggtgctttgaatgagttatttggttttggacttagtcttcaagagatagctaaattaggacatgaaattgaaattaaagttcagggtgcagctagtccaacagacacatatgtaagcacttttggcggtgtagttacaattccagaaagaagaaaacttaaaacaccagattgtggaatagtgattggtgatacaggcgtttttagttcaactaaagagttagtggctaatgtaagacagttaagagaatcttatcctgatcttattgagccattgatgacttcaataggaaaaataagcaggattggtgaacaacttgttttaagtggtgattacgcatctataggtagattaatgaatgtgaatcagggacttttggatgcattaggtgtaaatatattggaacttagccaacttatttatagtgcaagagcagctggtgcttttggcgcaaagataactggtgctggtggtggcggttgtatggttgcattaactgcacctgagaaatgtaaccaagtagcagaagctgttgcaggtgctggcggtaaggttacaataactaagcctactgaacagggattaaaagtagattaagcgccattcgatggtgtccgtccagataaaaataagaagcctgcatttgcaggcttcttatttttatgagcgaagcgaataagcgtcggaaaagcagactctatcattgatagagtttgaaactctatcattgatagagtataatatcttgtttaaacggtaccgaagtactaacaagtcaaattaaggagggaaaaatatggaagcaagaagatcagcaaattacgagccaaatagttgggattatgactatcttttatcttcagatacagatgaatctatagaagtatataaggataaagcaaagaaattggaagcagaagtaagaagagagataaataatgaaaaggcagaatttttaactcttcttgaacttatagataatgtgcaaaggcttggattaggatatagatttgaatcagatattagaggcgcattagatagatttgtatctagtggcggttttgatgctgttacaaaaacatcacttcatggaacagctcttagtttcagattattaaggcaacatggatttgaagtttctcaagaagctttttctggatttaaagaccaaaatggaaatttccttgaaaatcttaaagaagatataaaggcaattttatctttatatgaagcatcatttttggcattagaaggtgaaaacatattagatgaggcaaaagtttttgctataagtcatcttaaagaactttctgaagaaaagataggaaaagagttagcagagcaagtaaatcatgctcttgaattacctttacacagaagaacacaaagattagaagcagtgtggtctattgaagcatacagaaagaaagaagatgctaatcaggtattattagaattggcaattttagattataatatgatacagtctgtgtatcaaagggatttaagagagactagtagatggtggagaagagtaggattggctacaaaattgcattttgctagagacagacttattgaatcattttattgggctgttggtgtagcttttgaacctcagtatagcgattgtagaaacagtgtagcaaaaatgttcagttttgtaactataatagatgacatttatgatgtatatggaactcttgatgaattggaactttttacagacgcagtagaaagatgggatgtgaatgcaataaatgacttacctgattatatgaaattatgctttcttgcattatacaatactattaatgagattgcatatgataatttgaaagataaaggtgaaaatattcttccttatttaactaaagcttgggctgatttatgcaacgcattcttacaagaagctaaatggttgtataataaatcaacaccaacatttgatgattattttggtaacgcttggaaatctagctcaggaccattgcagttagtttttgcttattttgctgttgttcagaatataaagaaagaagaaatagagaacttacaaaaatatcatgatactatatcaaggccaagtcatatttttaggctttgtaatgacttagcatctgcttctgctgaaattgctagaggcgaaactgcaaattcagttagttgttacatgagaacaaagggtataagtgaagaattagcaactgagagcgtaatgaacttaatagatgaaacttggaaaaagatgaataaagagaaacttggcggtagtctttttgctaaaccatttgtagagactgcaataaatttggcaaggcaatcacattgtacatatcataatggtgatgctcacactagccctgatgagttaactagaaagagagttcttagtgttattacagaaccaatattgccttttgaaaggtaagcatgctctagaatagacaaatcgacatttaaaaaggaggacaatatatgatagaagtaacaacaccaggtaaattatttatagcaggtgaatacgcagtagttgaacctggacaccctgctataatagtagctgttgatcagtttgttacagtaacagttgaagagacaacagatgaaggatcaatacagtctgctcaatatagctcattgccaattagatggacaagaagaaatggtgagttagttttggatataagagaaaatccatttcattatgttcttgcagcaatacatttgactgagaaatacgctcaagaacaaaataaagaactttctttttatcatcttaaggttacttctgaattggattcttcaaatggtagaaaatacggattaggaagctcaggtgctgtaactgtaggtacagtaaaagcattaaatatattctatgacttaggattagaaaatgaagaaatttttaagctttctgcacttgctcatttagcagtgcaaggtaatggatcatgtggtgatattgctgcaagttgttatggtggctggatagcattcagtacttttgatcatgattgggtaaaccaaaaggtagcaactgaaacacttacagatttgcttgcaatggattggccagagttaatgatttttcctcttaaagtgccaaaacaattaagattattaattggctggactggtagtcctgcaagtacaagcgacttagttgatagagttcatcagtctaaagaagaaaagcaagcagcttatgagcaatttcttatgaaaagtaggttatgcgtggaaacaatgattaatggatttaatactggaaaaattagtgtgatacagaaacagataactaaaaacagacaacttcttgctgagttatcttctttaactggtgtagtaattgaaactgaagcattgaaaaacttatgcgatttagcagagtcatatactggtgctgcaaaatcatcaggtgctggtggtggcgattgtggaatagttatatttagacaaaagagtggcattttgcctcttatgactgcttgggaaaaagacggaattacacctcttccacttcatgtttatacatatggacagaaagaatgtaaagagaagcacgaaagtaaaaggtaagtcgagaaaaactaaaggtactaataaaaggaggttaaaagatgttatctggaaaagcaagggcacacacaaatatagctcttataaaatattggggtaaggctaatgaagaatatatattaccaatgaacagttcactttctttaacattagatgcattctatactgaaacaactgtgatatttgacgcacattattcagaagatgtttttatattagatggtatacttcaaaatgaaaaacagactaaaaaggtaaaagagtttttaaacttagtaaggcagcaagctgattgtacttggtttgctaaagttgaaagtcaaaattttgtgcctacagctgctggattggcttcaagtgcaagcggattggcagcattagcaggtgcatgtaacgtagctttaggacttaatttaagcgctaaggatctttcaagattagcaagaagaggctctggatcagcttgtagaagtatttttggcggttttgctcaatggaataagggacatagcgatgaaacatcttttgctgaaaacattccagcaaataattgggaaaatgaattagctatgcttttcatattgattaatgatggtgaaaaggatgtttctagtagagatggtatgaaaagaactgttgagacaagtagtttttatcagggttggcttgacaatgtagaaaaggatctttcacaggttcatgaagctattaaaacaaaagattttcctaggttaggtgaaattattgaggcaaatggattgagaatgcatggtactacattgggtgctgttcctccatttacatactggtcacctggatctttgcaagctatggcattagttagacaggctagagcaaagggtataccttgctacttcactatggatgcaggaccaaatgtaaaagtacttgtagagaagaaaaatttggaagcattaaagacttttcttagcgaacatttttctaaagaacaacttgtgcctgcttttgcaggtccaggtattgagttatttgaaactaaaggcatggacaaataagagctcgacaataaacacaggtaagtaaaggaggttaagaaatgcaaacagaacacgtaatattattaaacgcacaaggtgttcctactggaacacttgaaaagtatgctgcacatacagctgatacaagacttcatttagctttttcttcatggttattcaatgctaaaggacaacttcttgtaactagaagagcactttctaagaaagcttggcctggtgtttggactaacagtgtttgtggacatcctcagttaggtgaaagtaatgaagatgcagtaattagaaggtgcagatacgaattaggtgtagaaataactcctcctgagagtatatatcctgattttaggtatagagcaactgatccatctggcatagtagagaatgaagtatgtccagtgtttgcagcaagaactacatcagcattgcaaattaatgatgatgaagtaatggactatcagtggtgtgacttagcagatgttttacatggaattgacgcaactccatgggcttttagcccatggatggtgatgcaagctacaaatagagaagctagaaaaagattgtcagcttttacacagttgaaataagctagctgttcaaaacaatcgcaaattaaggaggctaataaatgataaacgcaaaacttttacaacttatggtagaacattcaaacgatggaattgttgtagctgaacaagaaggtaatgaaagcatattgatttatgttaatcctgcatttgaaaggttaacaggttattgtgcagacgatatattatatcaagatgcaaggtttcttcaaggtgaagatcacgatcagcctggaattgctattataagagaagctattagagaaggcagaccatgctgtcaggttttaagaaattatagaaaagacggatctttattttggaatgagcttagtataactccagtgcataatgaggctgatcaattaacttattacataggtatacaaagagatgtaacagctcaagttttcgctgaagaaagagtgagagaattggaagcagaagtagcagagcttagaagacaacagggacaggcaaagcattaagtccagatttaaat